European Patent Application EP 4 183 409 A1, published May 24, 2023. Title: VACCINE WITH IMPROVED IMMUNOGENICITY AGAINST MUTANT CORONAVIRUSES. Applicant: Charité - Universitätsmedizin Berlin. The sequence listing filed with the application follows.

SEQUENCE LISTING (15 sequences)

SEQ ID NO: 1 - protein, 1273 aa, Severe acute respiratory syndrome-related coronavirus
MFVFLVLLPLVSSQCVNLTTRTQLPPAYTNSFTRGVYYPDKVFRSSVLHSTQDLFLPFFSNVTWFHAIHVSGTNGTKRFDNPVLPFNDGVYFASTEKSNIIRGWIFGTTLDSKTQSLLIVNNATNVVIKVCEFQFCNDPFLGVYYHKNNKSWMESEFRVYSSANNCTFEYVSQPFLMDLEGKQGNFKNLREFVFKNIDGYFKIYSKHTPINLVRDLPQGFSALEPLVDLPIGINITRFQTLLALHRSYLTPGDSSSGWTAGAAAYYVGYLQPRTFLLKYNENGTITDAVDCALDPLSETKCTLKSFTVEKGIYQTSNFRVQPTESIVRFPNITNLCPFGEVFNATRFASVYAWNRKRISNCVADYSVLYNSASFSTFKCYGVSPTKLNDLCFTNVYADSFVIRGDEVRQIAPGQTGKIADYNYKLPDDFTGCVIAWNSNNLDSKVGGNYNYLYRLFRKSNLKPFERDISTEIYQAGSTPCNGVEGFNCYFPLQSYGFQPTNGVGYQPYRVVVLSFELLHAPATVCGPKKSTNLVKNKCVNFNFNGLTGTGVLTESNKKFLPFQQFGRDIADTTDAVRDPQTLEILDITPCSFGGVSVITPGTNTSNQVAVLYQDVNCTEVPVAIHADQLTPTWRVYSTGSNVFQTRAGCLIGAEHVNNSYECDIPIGAGICASYQTQTNSPRRARSVASQSIIAYTMSLGAENSVAYSNNSIAIPTNFTISVTTEILPVSMTKTSVDCTMYICGDSTECSNLLLQYGSFCTQLNRALTGIAVEQDKNTQEVFAQVKQIYKTPPIKDFGGFNFSQILPDPSKPSKRSFIEDLLFNKVTLADAGFIKQYGDCLGDIAARDLICAQKFNGLTVLPPLLTDEMIAQYTSALLAGTITSGWTFGAGAALQIPFAMQMAYRFNGIGVTQNVLYENQKLIANQFNSAIGKIQDSLSSTASALGKLQDVVNQNAQALNTLVKQLSSNFGAISSVLNDILSRLDKVEAEVQIDRLITGRLQSLQTYVTQQLIRAAEIRASANLAATKMSECVLGQSKRVDFCGKGYHLMSFPQSAPHGVVFLHVTYVPAQEKNFTTAPAICHDGKAHFPREGVFVSNGTHWFVTQRNFYEPQIITTDNTFVSGNCDVVIGIVNNTVYDPLQPELDSFKEELDKYFKNHTSPDVDLGDISGINASVVNIQKEIDRLNEVAKNLNESLIDLQELGKYEQYIKWPWYIWLGFIAGLIAIVMVTIMLCCMTSCCSCLKGCCSCGSCCKFDEDDSEPVLKGVKLHYT

SEQ ID NO: 2 - protein, 1270 aa, Severe acute respiratory syndrome-related coronavirus
  VARIANT (678)..(678): Position 678 can also be substituted with an R, wherein position 678 in B.1.1.7 (Alpha) refers to position 681 in WUHAN Sequence (SEQ ID No 1).
MFVFLVLLPLVSSQCVNLTTRTQLPPAYTNSFTRGVYYPDKVFRSSVLHSTQDLFLPFFSNVTWFHAISGTNGTKRFDNPVLPFNDGVYFASTEKSNIIRGWIFGTTLDSKTQSLLIVNNATNVVIKVCEFQFCNDPFLGVYHKNNKSWMESEFRVYSSANNCTFEYVSQPFLMDLEGKQGNFKNLREFVFKNIDGYFKIYSKHTPINLVRDLPQGFSALEPLVDLPIGINITRFQTLLALHRSYLTPGDSSSGWTAGAAAYYVGYLQPRTFLLKYNENGTITDAVDCALDPLSETKCTLKSFTVEKGIYQTSNFRVQPTESIVRFPNITNLCPFGEVFNATRFASVYAWNRKRISNCVADYSVLYNSASFSTFKCYGVSPTKLNDLCFTNVYADSFVIRGDEVRQIAPGQTGKIADYNYKLPDDFTGCVIAWNSNNLDSKVGGNYNYLYRLFRKSNLKPFERDISTEIYQAGSTPCNGVEGFNCYFPLQSYGFQPTYGVGYQPYRVVVLSFELLHAPATVCGPKKSTNLVKNKCVNFNFNGLTGTGVLTESNKKFLPFQQFGRDIDDTTDAVRDPQTLEILDITPCSFGGVSVITPGTNTSNQVAVLYQGVNCTEVPVAIHADQLTPTWRVYSTGSNVFQTRAGCLIGAEHVNNSYECDIPIGAGICASYQTQTNSHRRARSVASQSIIAYTMSLGAENSVAYSNNSIAIPINFTISVTTEILPVSMTKTSVDCTMYICGDSTECSNLLLQYGSFCTQLNRALTGIAVEQDKNTQEVFAQVKQIYKTPPIKDFGGFNFSQILPDPSKPSKRSFIEDLLFNKVTLADAGFIKQYGDCLGDIAARDLICAQKFNGLTVLPPLLTDEMIAQYTSALLAGTITSGWTFGAGAALQIPFAMQMAYRFNGIGVTQNVLYENQKLIANQFNSAIGKIQDSLSSTASALGKLQDVVNQNAQALNTLVKQLSSNFGAISSVLNDILARLDKVEAEVQIDRLITGRLQSLQTYVTQQLIRAAEIRASANLAATKMSECVLGQSKRVDFCGKGYHLMSFPQSAPHGVVFLHVTYVPAQEKNFTTAPAICHDGKAHFPREGVFVSNGTHWFVTQRNFYEPQIITTHNTFVSGNCDVVIGIVNNTVYDPLQPELDSFKEELDKYFKNHTSPDVDLGDISGINASVVNIQKEIDRLNEVAKNLNESLIDLQELGKYEQYIKWPWYIWLGFIAGLIAIVMVTIMLCCMTSCCSCLKGCCSCGSCCKFDEDDSEPVLKGVKLHYT

SEQ ID NO: 3 - protein, 1270 aa, Severe acute respiratory syndrome-related coronavirus
  VARIANT (481)..(481): Position 481 can also be substituted with an Q, wherein position 481 in B.1.351 (Beta) refers to position 681 in WUHAN Sequence (SEQ ID No 1).
MFVFLVLLPLVSSQCVNFTTRTQLPPAYTNSFTRGVYYPDKVFRSSVLHSTQDLFLPFFSNVTWFHAIHVSGTNGTKRFANPVLPFNDGVYFASTEKSNIIRGWIFGTTLDSKTQSLLIVNNATNVVIKVCEFQFCNDPFLGVYYHKNNKSWMESEFRVYSSANNCTFEYVSQPFLMDLEGKQGNFKNLREFVFKNIDGYFKIYSKHTPINLVRGLPQGFSALEPLVDLPIGINITRFQTLHRSYLTPGDSSSGWTAGAAAYYVGYLQPRTFLLKYNENGTITDAVDCALDPLSETKCTLKSFTVEKGIYQTSNFRVQPTESIVRFPNITNLCPFGEVFNATRFASVYAWNRKRISNCVADYSVLYNSASFSTFKCYGVSPTKLNDLCFTNVYADSFVIRGDEVRQIAPGQTGNIADYNYKLPDDFTGCVIAWNSNNLDSKVGGNYNYLYRLFRKSNLKPFERDISTEIYQAGSTPCNGVKGFNCYFPLQSYGFQPTYGVGYQPYRVVVLSFELLHAPATVCGPKKSTNLVKNKCVNFNFNGLTGTGVLTESNKKFLPFQQFGRDIADTTDAVRDPQTLEILDITPCSFGGVSVITPGTNTSNQVAVLYQGVNCTEVPVAIHADQLTPTWRVYSTGSNVFQTRAGCLIGAEHVNNSYECDIPIGAGICASYQTQTNSPRRARSVASQSIIAYTMSLGVENSVAYSNNSIAIPTNFTISVTTEILPVSMTKTSVDCTMYICGDSTECSNLLLQYGSFCTQLNRALTGIAVEQDKNTQEVFAQVKQIYKTPPIKDFGGFNFSQILPDPSKPSKRSFIEDLLFNKVTLADAGFIKQYGDCLGDIAARDLICAQKFNGLTVLPPLLTDEMIAQYTSALLAGTITSGWTFGAGAALQIPFAMQMAYRFNGIGVTQNVLYENQKLIANQFNSAIGKIQDSLSSTASALGKLQDVVNQNAQALNTLVKQLSSNFGAISSVLNDILSRLDKVEAEVQIDRLITGRLQSLQTYVTQQLIRAAEIRASANLAATKMSECVLGQSKRVDFCGKGYHLMSFPQSAPHGVVFLHVTYVPAQEKNFTTAPAICHDGKAHFPREGVFVSNGTHWFVTQRNFYEPQIITTDNTFVSGNCDVVIGIVNNTVYDPLQPELDSFKEELDKYFKNHTSPDVDLGDISGINASVVNIQKEIDRLNEVAKNLNESLIDLQELGKYEQYIKWPWYIWLGFIAGLIAIVMVTIMLCCMTSCCSCLKGCCSCGSCCKFDEDDSEPVLKGVKLHYT

SEQ ID NO: 4 - protein, 1271 aa, Severe acute respiratory syndrome-related coronavirus
  VARIANT (450)..(450): Position 450 can also be substituted with an Q, wherein position 450 in B.1.617.2 (Delta) refers to position 452 in WUHAN Sequence (SEQ ID No 1).
  VARIANT (679)..(679): Position 679 can also be substituted with an H, wherein position 679 in B.1.617.2 (Delta) refers to position 681 in WUHAN Sequence (SEQ ID No 1).
MFVFLVLLPLVSSQCVNLRTRTQLPPAYTNSFTRGVYYPDKVFRSSVLHSTQDLFLPFFSNVTWFHAIHVSGTNGTKRFDNPVLPFNDGVYFASTEKSNIIRGWIFGTTLDSKTQSLLIVNNATNVVIKVCEFQFCNDPFLGVYYHKNNKSWMESEVYSSANNCTFEYVSQPFLMDLEGKQGNFKNLREFVFKNIDGYFKIYSKHTPINLVRDLPQGFSALEPLVDLPIGINITRFQTLLALHRSYLTPGDSSSGWTAGAAAYYVGYLQPRTFLLKYNENGTITDAVDCALDPLSETKCTLKSFTVEKGIYQTSNFRVQPTESIVRFPNITNLCPFGEVFNATRFASVYAWNRKRISNCVADYSVLYNSASFSTFKCYGVSPTKLNDLCFTNVYADSFVIRGDEVRQIAPGQTGKIADYNYKLPDDFTGCVIAWNSNNLDSKVGGNYNYRYRLFRKSNLKPFERDISTEIYQAGSKPCNGVEGFNCYFPLQSYGFQPTNGVGYQPYRVVVLSFELLHAPATVCGPKKSTNLVKNKCVNFNFNGLTGTGVLTESNKKFLPFQQFGRDIADTTDAVRDPQTLEILDITPCSFGGVSVITPGTNTSNQVAVLYQGVNCTEVPVAIHADQLTPTWRVYSTGSNVFQTRAGCLIGAEHVNNSYECDIPIGAGICASYQTQTNSRRRARSVASQSIIAYTMSLGAENSVAYSNNSIAIPTNFTISVTTEILPVSMTKTSVDCTMYICGDSTECSNLLLQYGSFCTQLNRALTGIAVEQDKNTQEVFAQVKQIYKTPPIKDFGGFNFSQILPDPSKPSKRSFIEDLLFNKVTLADAGFIKQYGDCLGDIAARDLICAQKFNGLTVLPPLLTDEMIAQYTSALLAGTITSGWTFGAGAALQIPFAMQMAYRFNGIGVTQNVLYENQKLIANQFNSAIGKIQDSLSSTASALGKLQNVVNQNAQALNTLVKQLSSNFGAISSVLNDILSRLDKVEAEVQIDRLITGRLQSLQTYVTQQLIRAAEIRASANLAATKMSECVLGQSKRVDFCGKGYHLMSFPQSAPHGVVFLHVTYVPAQEKNFTTAPAICHDGKAHFPREGVFVSNGTHWFVTQRNFYEPQIITTDNTFVSGNCDVVIGIVNNTVYDPLQPELDSFKEELDKYFKNHTSPDVDLGDISGINASVVNIQKEIDRLNEVAKNLNESLIDLQELGKYEQYIKWPWYIWLGFIAGLIAIVMVTIMLCCMTSCCSCLKGCCSCGSCCKFDEDDSEPVLKGVKLHYT

SEQ ID NO: 5 - protein, 1273 aa, Severe acute respiratory syndrome-related coronavirus
  VARIANT (484)..(484): Position 484 can also be substituted with an Q.
MFVFLVLLPLVSSQCVNFTNRTQLPSAYTNSFTRGVYYPDKVFRSSVLHSTQDLFLPFFSNVTWFHAIHVSGTNGTKRFDNPVLPFNDGVYFASTEKSNIIRGWIFGTTLDSKTQSLLIVNNATNVVIKVCEFQFCNYPFLGVYYHKNNKSWMESEFRVYSSANNCTFEYVSQPFLMDLEGKQGNFKNLSEFVFKNIDGYFKIYSKHTPINLVRDLPQGFSALEPLVDLPIGINITRFQTLLALHRSYLTPGDSSSGWTAGAAAYYVGYLQPRTFLLKYNENGTITDAVDCALDPLSETKCTLKSFTVEKGIYQTSNFRVQPTESIVRFPNITNLCPFGEVFNATRFASVYAWNRKRISNCVADYSVLYNSASFSTFKCYGVSPTKLNDLCFTNVYADSFVIRGDEVRQIAPGQTGTIADYNYKLPDDFTGCVIAWNSNNLDSKVGGNYNYLYRLFRKSNLKPFERDISTEIYQAGSTPCNGVKGFNCYFPLQSYGFQPTYGVGYQPYRVVVLSFELLHAPATVCGPKKSTNLVKNKCVNFNFNGLTGTGVLTESNKKFLPFQQFGRDIADTTDAVRDPQTLEILDITPCSFGGVSVITPGTNTSNQVAVLYQGVNCTEVPVAIHADQLTPTWRVYSTGSNVFQTRAGCLIGAEYVNNSYECDIPIGAGICASYQTQTNSPRRARSVASQSIIAYTMSLGAENSVAYSNNSIAIPTNFTISVTTEILPVSMTKTSVDCTMYICGDSTECSNLLLQYGSFCTQLNRALTGIAVEQDKNTQEVFAQVKQIYKTPPIKDFGGFNFSQILPDPSKPSKRSFIEDLLFNKVTLADAGFIKQYGDCLGDIAARDLICAQKFNGLTVLPPLLTDEMIAQYTSALLAGTITSGWTFGAGAALQIPFAMQMAYRFNGIGVTQNVLYENQKLIANQFNSAIGKIQDSLSSTASALGKLQDVVNQNAQALNTLVKQLSSNFGAISSVLNDILSRLDKVEAEVQIDRLITGRLQSLQTYVTQQLIRAAEIRASANLAAIKMSECVLGQSKRVDFCGKGYHLMSFPQSAPHGVVFLHVTYVPAQEKNFTTAPAICHDGKAHFPREGVFVSNGTHWFVTQRNFYEPQIITTDNTFVSGNCDVVIGIVNNTVYDPLQPELDSFKEELDKYFKNHTSPDVDLGDISGINASFVNIQKEIDRLNEVAKNLNESLIDLQELGKYEQYIKWPWYIWLGFIAGLIAIVMVTIMLCCMTSCCSCLKGCCSCGSCCKFDEDDSEPVLKGVKLHYT

SEQ ID NO: 6 - protein, 1266 aa, Severe acute respiratory syndrome-related coronavirus
  VARIANT (445)..(445): Position 445 can also be substituted with an R, wherein position 445 in C.37 Lambda refers to position 452 in WUHAN Sequence (SEQ ID No 1).
MFVFLVLLPLVSSQCVNLTTRTQLPPAYTNSFTRGVYYPDKVFRSSVLHSTQDLFLPFFSNVTWFHAIHVSGTNVIKRFDNPVLPFNDGVYFASTEKSNIIRGWIFGTTLDSKTQSLLIVNNATNVVIKVCEFQFCNDPFLGVYYHKNNKSWMESEFRVYSSANNCTFEYVSQPFLMDLEGKQGNFKNLREFVFKNIDGYFKIYSKHTPINLVRDLPQGFSALEPLVDLPIGINITRFQTLLALHNSSSGWTAGAAAYYVGYLQPRTFLLKYNENGTITDAVDCALDPLSETKCTLKSFTVEKGIYQTSNFRVQPTESIVRFPNITNLCPFGEVFNATRFASVYAWNRKRISNCVADYSVLYNSASFSTFKCYGVSPTKLNDLCFTNVYADSFVIRGDEVRQIAPGQTGKIADYNYKLPDDFTGCVIAWNSNNLDSKVGGNYNYQYRLFRKSNLKPFERDISTEIYQAGSTPCNGVEGFNCYSPLQSYGFQPTNGVGYQPYRVVVLSFELLHAPATVCGPKKSTNLVKNKCVNFNFNGLTGTGVLTESNKKFLPFQQFGRDIADTTDAVRDPQTLEILDITPCSFGGVSVITPGTNTSNQVAVLYQGVNCTEVPVAIHADQLTPTWRVYSTGSNVFQTRAGCLIGAEHVNNSYECDIPIGAGICASYQTQTNSPRRARSVASQSIIAYTMSLGAENSVAYSNNSIAIPTNFTISVTTEILPVSMTKTSVDCTMYICGDSTECSNLLLQYGSFCTQLNRALTGIAVEQDKNTQEVFAQVKQIYKTPPIKDFGGFNFSQILPDPSKPSKRSFIEDLLFNKVTLADAGFIKQYGDCLGDIAARDLICAQKFNGLNVLPPLLTDEMIAQYTSALLAGTITSGWTFGAGAALQIPFAMQMAYRFNGIGVTQNVLYENQKLIANQFNSAIGKIQDSLSSTASALGKLQDVVNQNAQALNTLVKQLSSNFGAISSVLNDILSRLDKVEAEVQIDRLITGRLQSLQTYVTQQLIRAAEIRASANLAATKMSECVLGQSKRVDFCGKGYHLMSFPQSAPHGVVFLHVTYVPAQEKNFTTAPAICHDGKAHFPREGVFVSNGTHWFVTQRNFYEPQIITTDNTFVSGNCDVVIGIVNNTVYDPLQPELDSFKEELDKYFKNHTSPDVDLGDISGINASVVNIQKEIDRLNEVAKNLNESLIDLQELGKYEQYIKWPWYIWLGFIAGLIAIVMVTIMLCCMTSCCSCLKGCCSCGSCCKFDEDDSEPVLKGVKLHYT

SEQ ID NO: 7 - protein, 1270 aa, Artificial Sequence
  SARS-CoV-2 spike like protein
MFVFLVLLPLVSSQCVNFTNRTQLPSAYTNSFTRGVYYPDKVFRSSVLHSTQDLFLPFFSNVTWFHAISGTNGTKRFDNPVLPFNDGVYFASTEKSNIIRGWIFGTTLDSKTQSLLIVNNATNVVIKVCEFQFCNYPFLGVYHKNNKSWMESEFRVYSSANNCTFEYVSQPFLMDLEGKQGNFKNLSEFVFKNIDGYFKIYSKHTPINLVRDLPQGFSALEPLVDLPIGINITRFQTLLALHRSYLTPGDSSSGWTAGAAAYYVGYLQPRTFLLKYNENGTITDAVDCALDPLSETKCTLKSFTVEKGIYQTSNFRVQPTESIVRFPNITNLCPFGEVFNATRFASVYAWNRKRISNCVADYSVLYNSASFSTFKCYGVSPTKLNDLCFTNVYADSFVIRGDEVRQIAPGQTGTIADYNYKLPDDFTGCVIAWNSNNLDSKVGGNYNYLYRLFRKSNLKPFERDISTEIYQAGSTPCNGVKGFNCYFPLQSYGFQPTYGVGYQPYRVVVLSFELLHAPATVCGPKKSTNLVKNKCVNFNFNGLTGTGVLTESNKKFLPFQQFGRDIDDTTDAVRDPQTLEILDITPCSFGGVSVITPGTNTSNQVAVLYQGVNCTEVPVAIHADQLTPTWRVYSTGSNVFQTRAGCLIGAEYVNNSYECDIPIGAGICASYQTQTNSHRRARSVASQSIIAYTMSLGAENSVAYSNNSIAIPINFTISVTTEILPVSMTKTSVDCTMYICGDSTECSNLLLQYGSFCTQLNRALTGIAVEQDKNTQEVFAQVKQIYKTPPIKDFGGFNFSQILPDPSKPSKRSPIEDLLFNKVTLADAGFIKQYGDCLGDIAARDLICAQKFNGLTVLPPLLTDEMIAQYTSALLAGTITSGWTFGAGPALQIPFPMQMAYRFNGIGVTQNVLYENQKLIANQFNSAIGKIQDSLSSTPSALGKLQDVVNQNAQALNTLVKQLSSNFGAISSVLNDILARLDPPEAEVQIDRLITGRLQSLQTYVTQQLIRAAEIRASANLAAIKMSECVLGQSKRVDFCGKGYHLMSFPQSAPHGVVFLHVTYVPAQEKNFTTAPAICHDGKAHFPREGVFVSNGTHWFVTQRNFYEPQIITTHNTFVSGNCDVVIGIVNNTVYDPLQPELDSFKEELDKYFKNHTSPDVDLGDISGINASVVNIQKEIDRLNEVAKNLNESLIDLQELGKYEQYIKWPWYIWLGFIAGLIAIVMVTIMLCCMTSCCSCLKGCCSCGSCCKFDEDDSEPVLKGVKLHYT

SEQ ID NO: 8 - protein, 1270 aa, Artificial Sequence; identical to SEQ ID NO: 7
  SARS-CoV-2 spike like protein

SEQ ID NO: 9 - protein, 1261 aa, Artificial Sequence
  SARS-CoV-2 spike like protein
MFVFLVLLPLVSSQCVNFRNRTQLPSAYTNSFTRGVYYPDKVFRSSVLHSTQDLFLPFFSNVTWFHAISGTNVIKRFDNPVLPFNDGVYFASTEKSNIIRGWIFGTTLDSKTQSLLIVNNATNVVIKVCEFQFCNYPFLGVYHKNNKSWMESGVYSSANNCTFEYVSQPFLMDLEGKQGNFKNLSEFVFKNIDGYFKIYSKHTPINLVRGLPQGFSALEPLVDLPIGINITRFQTLLALHNSSSGWTAGAAAYYVGYLQPRTFLLKYNENGTITDAVDCALDPLSETKCTLKSFTVEKGIYQTSNFRVQPTESIVRFPNITNLCPFGEVFNATRFASVYAWNRKRISNCVADYSVLYNSASFSTFKCYGVSPTKLNDLCFTNVYADSFVIRGDEVRQIAPGQTGTIADYNYKLPDDFTGCVIAWNSNNLDSKVGGNYNYRYRLFRKSNLKPFERDISTEIYQAGSKPCNGVQGFNCYSPLQSYGFQPTYGVGYQPYRVVVLSFELLHAPATVCGPKKSTNLVKNKCVNFNFNGLTGTGVLTESNKKFLPFQQFGRDIADTTDAVRDPQTLEILDITPCSFGGVSVITPGTNTSNQVAVLYQGVNCTEVPVAIHADQLTPTWRVYSTGSNVFQTRAGCLIGAEYVNNSYECDIPIGAGICASYQTQTNSRRRARSVASQSIIAYTMSLGAENSVAYSNNSIAIPINFTISVTTEILPVSMTKTSVDCTMYICGDSTECSNLLLQYGSFCTQLNRALTGIAVEQDKNTQEVFAQVKQIYKTPPIKDFGGFNFSQILPDPSKPSKRSPIEDLLFNKVTLADAGFIKQYGDCLGDIAARDLICAQKFNGLNVLPPLLTDEMIAQYTSALLAGTITSGWTFGAGPALQIPFPMQMAYRFNGIGVTQNVLYENQKLIANQFNSAIGKIQDSLSSTPSALGKLQNVVNQNAQALNTLVKQLSSNFGAISSVLNDILARLDPPEAEVQIDRLITGRLQSLQTYVTQQLIRAAEIRASANLAAIKMSECVLGQSKRVDFCGKGYHLMSFPQSAPHGVVFLHVTYVPAQEKNFTTAPAICHDGKAHFPREGVFVSNGTHWFVTQRNFYEPQIITTHNTFVSGNCDVVIGIVNNTVYDPLQPELDSFKEELDKYFKNHTSPDVDLGDISGINASFVNIQKEIDRLNEVAKNLNESLIDLQELGKYEQYIKWPWYIWLGFIAGLIAIVMVTIMLCCMTSCCSCLKGCCSCGSCCKFDEDDSEPVLKGVKLHYT

SEQ ID NO: 10 - protein, 1268 aa, Artificial Sequence
  SARS-CoV-2 spike like protein
MFVFLVLLPLVSSQCVNFRNRTQLPSAYTNSFTRGVYYPDKVFRSSVLHSTQDLFLPFFSNVTWFHAISGTNGTKRFDNPVLPFNDGVYFASTEKSNIIRGWIFGTTLDSKTQSLLIVNNATNVVIKVCEFQFCNYPFLGVYHKNNKSWMESEVYSSANNCTFEYVSQPFLMDLEGKQGNFKNLSEFVFKNIDGYFKIYSKHTPINLVRDLPQGFSALEPLVDLPIGINITRFQTLLALHRSYLTPGDSSSGWTAGAAAYYVGYLQPRTFLLKYNENGTITDAVDCALDPLSETKCTLKSFTVEKGIYQTSNFRVQPTESIVRFPNITNLCPFGEVFNATRFASVYAWNRKRISNCVADYSVLYNSASFSTFKCYGVSPTKLNDLCFTNVYADSFVIRGDEVRQIAPGQTGTIADYNYKLPDDFTGCVIAWNSNNLDSKVGGNYNYRYRLFRKSNLKPFERDISTEIYQAGSKPCNGVKGFNCYFPLQSYGFQPTYGVGYQPYRVVVLSFELLHAPATVCGPKKSTNLVKNKCVNFNFNGLTGTGVLTESNKKFLPFQQFGRDIDDTTDAVRDPQTLEILDITPCSFGGVSVITPGTNTSNQVAVLYQGVNCTEVPVAIHADQLTPTWRVYSTGSNVFQTRAGCLIGAEYVNNSYECDIPIGAGICASYQTQTNSHRRARSVASQSIIAYTMSLGAENSVAYSNNSIAIPINFTISVTTEILPVSMTKTSVDCTMYICGDSTECSNLLLQYGSFCTQLNRALTGIAVEQDKNTQEVFAQVKQIYKTPPIKDFGGFNFSQILPDPSKPSKRSPIEDLLFNKVTLADAGFIKQYGDCLGDIAARDLICAQKFNGLTVLPPLLTDEMIAQYTSALLAGTITSGWTFGAGPALQIPFPMQMAYRFNGIGVTQNVLYENQKLIANQFNSAIGKIQDSLSSTPSALGKLQNVVNQNAQALNTLVKQLSSNFGAISSVLNDILARLDPPEAEVQIDRLITGRLQSLQTYVTQQLIRAAEIRASANLAAIKMSECVLGQSKRVDFCGKGYHLMSFPQSAPHGVVFLHVTYVPAQEKNFTTAPAICHDGKAHFPREGVFVSNGTHWFVTQRNFYEPQIITTHNTFVSGNCDVVIGIVNNTVYDPLQPELDSFKEELDKYFKNHTSPDVDLGDISGINASVVNIQKEIDRLNEVAKNLNESLIDLQELGKYEQYIKWPWYIWLGFIAGLIAIVMVTIMLCCMTSCCSCLKGCCSCGSCCKFDEDDSEPVLKGVKLHYT

SEQ ID NO: 11 - protein, 1271 aa, Severe acute respiratory syndrome-related coronavirus
MFVFLVLLPLVSSQCVNLRTRTQLPPAYTNSFTRGVYYPDKVFRSSVLHSTQDLFLPFFSNVTWFHAIHVSGTNGTKRFDNPVLPFNDGVYFASTEKSNIIRGWIFGTTLDSKTQSLLIVNNATNVVIKVCEFQFCNDPFLGVYYHKNNKSWMESEVYSSANNCTFEYVSQPFLMDLEGKQGNFKNLREFVFKNIDGYFKIYSKHTPINLVRDLPQGFSALEPLVDLPIGINITRFQTLLALHRSYLTPGDSSSGWTAGAAAYYVGYLQPRTFLLKYNENGTITDAVDCALDPLSETKCTLKSFTVEKGIYQTSNFRVQPTESIVRFPNITNLCPFGEVFNATRFASVYAWNRKRISNCVADYSVLYNSASFSTFKCYGVSPTKLNDLCFTNVYADSFVIRGDEVRQIAPGQTGNIADYNYKLPDDFTGCVIAWNSNNLDSKVGGNYNYRYRLFRKSNLKPFERDISTEIYQAGSKPCNGVEGFNCYFPLQSYGFQPTNGVGYQPYRVVVLSFELLHAPATVCGPKKSTNLVKNKCVNFNFNGLTGTGVLTESNKKFLPFQQFGRDIADTTDAVRDPQTLEILDITPCSFGGVSVITPGTNTSNQVAVLYQGVNCTEVPVAIHADQLTPTWRVYSTGSNVFQTRAGCLIGAEHVNNSYECDIPIGAGICASYQTQTNSRRRARSVASQSIIAYTMSLGAENSVAYSNNSIAIPTNFTISVTTEILPVSMTKTSVDCTMYICGDSTECSNLLLQYGSFCTQLNRALTGIAVEQDKNTQEVFAQVKQIYKTPPIKDFGGFNFSQILPDPSKPSKRSFIEDLLFNKVTLADAGFIKQYGDCLGDIAARDLICAQKFNGLTVLPPLLTDEMIAQYTSALLAGTITSGWTFGAGAALQIPFAMQMAYRFNGIGVTQNVLYENQKLIANQFNSAIGKIQDSLSSTASALGKLQNVVNQNAQALNTLVKQLSSNFGAISSVLNDILSRLDKVEAEVQIDRLITGRLQSLQTYVTQQLIRAAEIRASANLAATKMSECVLGQSKRVDFCGKGYHLMSFPQSAPHGVVFLHVTYVPAQEKNFTTAPAICHDGKAHFPREGVFVSNGTHWFVTQRNFYEPQIITTDNTFVSGNCDVVIGIVNNTVYDPLQPELDSFKEELDKYFKNHTSPDVDLGDISGINASVVNIQKEIDRLNEVAKNLNESLIDLQELGKYEQYIKWPWYIWLGFIAGLIAIVMVTIMLCCMTSCCSCLKGCCSCGSCCKFDEDDSEPVLKGVKLHYT

SEQ ID NO: 12 - DNA, 3822 bp, Severe acute respiratory syndrome-related coronavirus
atgtttgtttttcttgttttattgccactagtctctagtcagtgtgttaatcttacaaccagaactcaattaccccctgcatacactaattctttcacacgtggtgtttattaccctgacaaagttttcagatcctcagttttacattcaactcaggacttgttcttacctttcttttccaatgttacttggttccatgctatacatgtctctgggaccaatggtactaagaggtttgataaccctgtcctaccatttaatgatggtgtttattttgcttccactgagaagtctaacataataagaggctggatttttggtactactttagattcgaagacccagtccctacttattgttaataacgctactaatgttgttattaaagtctgtgaatttcaattttgtaatgatccatttttgggtgtttattaccacaaaaacaacaaaagttggatggaaagtgagttcagagtttattctagtgcgaataattgcacttttgaatatgtctctcagccttttcttatggaccttgaaggaaaacagggtaatttcaaaaatcttagggaatttgtgtttaagaatattgatggttattttaaaatatattctaagcacacgcctattaatttagtgcgtgatctccctcagggtttttcggctttagaaccattggtagatttgccaataggtattaacatcactaggtttcaaactttacttgctttacatagaagttatttgactcctggtgattcttcttcaggttggacagctggtgctgcagcttattatgtgggttatcttcaacctaggacttttctattaaaatataatgaaaatggaaccattacagatgctgtagactgtgcacttgaccctctctcagaaacaaagtgtacgttgaaatccttcactgtagaaaaaggaatctatcaaacttctaactttagagtccaaccaacagaatctattgttagatttcctaatattacaaacttgtgcccttttggtgaagtttttaacgccaccagatttgcatctgtttatgcttggaacaggaagagaatcagcaactgtgttgctgattattctgtcctatataattccgcatcattttccacttttaagtgttatggagtgtctcctactaaattaaatgatctctgctttactaatgtctatgcagattcatttgtaattagaggtgatgaagtcagacaaatcgctccagggcaaactggaaagattgctgattataattataaattaccagatgattttacaggctgcgttatagcttggaattctaacaatcttgattctaaggttggtggtaattataattacctgtatagattgtttaggaagtctaatctcaaaccttttgagagagatatttcaactgaaatctatcaggccggtagcacaccttgtaatggtgttgaaggttttaattgttactttcctttacaatcatatggtttccaacccactaatggtgttggttaccaaccatacagagtagtagtactttcttttgaacttctacatgcaccagcaactgtttgtggacctaaaaagtctactaatttggttaaaaacaaatgtgtcaatttcaacttcaatggtttaacaggcacaggtgttcttactgagtctaacaaaaagtttctgcctttccaacaatttggcagagacattgctgacactactgatgctgtccgtgatccacagacacttgagattcttgacattacaccatgttcttttggtggtgtcagtgttataacaccaggaacaaatacttctaaccaggttgctgttctttatcaggatgttaactgcacagaagtccctgttgctattcatgcagatcaacttactcctacttggcgtgtttattctacaggttctaatgtttttcaaacacgtgcaggctgtttaataggggctgaacatgtcaacaactcatatgagtgtgacatacccattggtgcaggtatatgcgctagttatcagactcagactaattctcctcggcgggcacgtagtgtagctagtcaatccatcattgcctacactatgtcacttggtgcagaaaattcagttgcttactctaataactctattgccatacccacaaattttactattagtgttaccacagaaattctaccagtgtctatgaccaagacatcagtagattgtacaatgtacatttgtggtgattcaactgaatgcagcaatcttttgttgcaatatggcagtttttgtacacaattaaaccgtgctttaactggaatagctgttgaacaagacaaaaacacccaagaagtttttgcacaagtcaaacaaatttacaaaacaccaccaattaaagattttggtggttttaatttttcacaaatattaccagatccatcaaaaccaagcaagaggtcatttattgaagatctacttttcaacaaagtgacacttgcagatgctggcttcatcaaacaatatggtgattgccttggtgatattgctgctagagacctcatttgtgcacaaaagtttaacggccttactgttttgccacctttgctcacagatgaaatgattgctcaatacacttctgcactgttagcgggtacaatcacttctggttggacctttggtgcaggtgctgcattacaaataccatttgctatgcaaatggcttataggtttaatggtattggagttacacagaatgttctctatgagaaccaaaaattgattgccaaccaatttaatagtgctattggcaaaattcaagactcactttcttccacagcaagtgcacttggaaaacttcaagatgtggtcaaccaaaatgcacaagctttaaacacgcttgttaaacaacttagctccaattttggtgcaatttcaagtgttttaaatgatatcctttcacgtcttgacaaagttgaggctgaagtgcaaattgataggttgatcacaggcagacttcaaagtttgcagacatatgtgactcaacaattaattagagctgcagaaatcagagcttctgctaatcttgctgctactaaaatgtcagagtgtgtacttggacaatcaaaaagagttgatttttgtggaaagggctatcatcttatgtccttccctcagtcagcacctcatggtgtagtcttcttgcatgtgacttatgtccctgcacaagaaaagaacttcacaactgctcctgccatttgtcatgatggaaaagcacactttcctcgtgaaggtgtctttgtttcaaatggcacacactggtttgtaacacaaaggaatttttatgaaccacaaatcattactacagacaacacatttgtgtctggtaactgtgatgttgtaataggaattgtcaacaacacagtttatgatcctttgcaacctgaattagactcattcaaggaggagttagataaatattttaagaatcatacatcaccagatgttgatttaggtgacatctctggcattaatgcttcagttgtaaacattcaaaaagaaattgaccgcctcaatgaggttgccaagaatttaaatgaatctctcatcgatctccaagaacttggaaagtatgagcagtatataaaatggccatggtacatttggctaggttttatagctggcttgattgccatagtaatggtgacaattatgctttgctgtatgaccagttgctgtagttgtctcaagggctgttgttcttgtggatcctgctgcaaatttgatgaagacgactctgagccagtgctcaaaggagtcaaattacattacacataa

SEQ ID NO: 13 - DNA, 3813 bp, Severe acute respiratory syndrome-related coronavirus
atgtttgtttttcttgttttattgccactagtctctagtcagtgtgttaatcttacaaccagaactcaattaccccctgcatacactaattctttcacacgtggtgtttattaccctgacaaagttttcagatcctcagttttacattcaactcaggacttgttcttacctttcttttccaatgttacttggttccatgctatctctgggaccaatggtactaagaggtttgataaccctgtcctaccatttaatgatggtgtttattttgcttccactgagaagtctaacataataagaggctggatttttggtactactttagattcgaagacccagtccctacttattgttaataacgctactaatgttgttattaaagtctgtgaatttcaattttgtaatgatccatttttgggtgtttaccacaaaaacaacaaaagttggatggaaagtgagttcagagtttattctagtgcgaataattgcacttttgaatatgtctctcagccttttcttatggaccttgaaggaaaacagggtaatttcaaaaatcttagggaatttgtgtttaagaatattgatggttattttaaaatatattctaagcacacgcctattaatttagtgcgtgatctccctcagggtttttcggctttagaaccattggtagatttgccaataggtattaacatcactaggtttcaaactttacttgctttacatagaagttatttgactcctggtgattcttcttcaggttggacagctggtgctgcagcttattatgtgggttatcttcaacctaggacttttctattaaaatataatgaaaatggaaccattacagatgctgtagactgtgcacttgaccctctctcagaaacaaagtgtacgttgaaatccttcactgtagaaaaaggaatctatcaaacttctaactttagagtccaaccaacagaatctattgttagatttcctaatattacaaacttgtgcccttttggtgaagtttttaacgccaccagatttgcatctgtttatgcttggaacaggaagagaatcagcaactgtgttgctgattattctgtcctatataattccgcatcattttccacttttaagtgttatggagtgtctcctactaaattaaatgatctctgctttactaatgtctatgcagattcatttgtaattagaggtgatgaagtcagacaaatcgctccagggcaaactggaaagattgctgattataattataaattaccagatgattttacaggctgcgttatagcttggaattctaacaatcttgattctaaggttggtggtaattataattacctgtatagattgtttaggaagtctaatctcaaaccttttgagagagatatttcaactgaaatctatcaggccggtagcacaccttgtaatggtgttgaaggttttaattgttactttcctttacaatcatatggtttccaacccacttatggtgttggttaccaaccatacagagtagtagtactttcttttgaacttctacatgcaccagcaactgtttgtggacctaaaaagtctactaatttggttaaaaacaaatgtgtcaatttcaacttcaatggtttaacaggcacaggtgttcttactgagtctaacaaaaagtttctgcctttccaacaatttggcagagacattgatgacactactgatgctgtccgtgatccacagacacttgagattcttgacattacaccatgttcttttggtggtgtcagtgttataacaccaggaacaaatacttctaaccaggttgctgttctttatcagggtgttaactgcacagaagtccctgttgctattcatgcagatcaacttactcctacttggcgtgtttattctacaggttctaatgtttttcaaacacgtgcaggctgtttaataggggctgaacatgtcaacaactcatatgagtgtgacatacccattggtgcaggtatatgcgctagttatcagactcagactaattctcatcggcgggcacgtagtgtagctagtcaatccatcattgcctacactatgtcacttggtgcagaaaattcagttgcttactctaataactctattgccatacccataaattttactattagtgttaccacagaaattctaccagtgtctatgaccaagacatcagtagattgtacaatgtacatttgtggtgattcaactgaatgcagcaatcttttgttgcaatatggcagtttttgtacacaattaaaccgtgctttaactggaatagctgttgaacaagacaaaaacacccaagaagtttttgcacaagtcaaacaaatttacaaaacaccaccaattaaagattttggtggttttaatttttcacaaatattaccagatccatcaaaaccaagcaagaggtcatttattgaagatctacttttcaacaaagtgacacttgcagatgctggcttcatcaaacaatatggtgattgccttggtgatattgctgctagagacctcatttgtgcacaaaagtttaacggccttactgttttgccacctttgctcacagatgaaatgattgctcaatacacttctgcactgttagcgggtacaatcacttctggttggacctttggtgcaggtgctgcattacaaataccatttgctatgcaaatggcttataggtttaatggtattggagttacacagaatgttctctatgagaaccaaaaattgattgccaaccaatttaatagtgctattggcaaaattcaagactcactttcttccacagcaagtgcacttggaaaacttcaagatgtggtcaaccaaaatgcacaagctttaaacacgcttgttaaacaacttagctccaattttggtgcaatttcaagtgttttaaatgatatccttgcacgtcttgacaaagttgaggctgaagtgcaaattgataggttgatcacaggcagacttcaaagtttgcagacatatgtgactcaacaattaattagagctgcagaaatcagagcttctgctaatcttgctgctactaaaatgtcagagtgtgtacttggacaatcaaaaagagttgatttttgtggaaagggctatcatcttatgtccttccctcagtcagcacctcatggtgtagtcttcttgcatgtgacttatgtccctgcacaagaaaagaacttcacaactgctcctgccatttgtcatgatggaaaagcacactttcctcgtgaaggtgtctttgtttcaaatggcacacactggtttgtaacacaaaggaatttttatgaaccacaaatcattactacacacaacacatttgtgtctggtaactgtgatgttgtaataggaattgtcaacaacacagtttatgatcctttgcaacctgaattagactcattcaaggaggagttagataaatattttaagaatcatacatcaccagatgttgatttaggtgacatctctggcattaatgcttcagttgtaaacattcaaaaagaaattgaccgcctcaatgaggttgccaagaatttaaatgaatctctcatcgatctccaagaacttggaaagtatgagcagtatataaaatggccatggtacatttggctaggttttatagctggcttgattgccatagtaatggtgacaattatgctttgctgtatgaccagttgctgtagttgtctcaagggctgttgttcttgtggatcctgctgcaaatttgatgaagacgactctgagccagtgctcaaaggagtcaaattacattacacataa

SEQ ID NO: 14 - DNA, 3813 bp, Severe acute respiratory syndrome-related coronavirus
atgtttgtttttcttgttttattgccactagtctctagtcagtgtgttaattttacaaccagaactcaattaccccctgcatacactaattctttcacacgtggtgtttattaccctgacaaagttttcagatcctcagttttacattcaactcaggacttgttcttacctttcttttccaatgttacttggttccatgctatacatgtctctgggaccaatggtactaagaggtttgctaaccctgtcctaccatttaatgatggtgtttattttgcttccactgagaagtctaacataataagaggctggatttttggtactactttagattcgaagacccagtccctacttattgttaataacgctactaatgttgttattaaagtctgtgaatttcaattttgtaatgatccatttttgggtgtttattaccacaaaaacaacaaaagttggatggaaagtgagttcagagtttattctagtgcgaataattgcacttttgaatatgtctctcagccttttcttatggaccttgaaggaaaacagggtaatttcaaaaatcttagggaatttgtgtttaagaatattgatggttattttaaaatatattctaagcacacgcctattaatttagtgcgtggtctccctcagggtttttcggctttagaaccattggtagatttgccaataggtattaacatcactaggtttcaaactttacatagaagttatttgactcctggtgattcttcttcaggttggacagctggtgctgcagcttattatgtgggttatcttcaacctaggacttttctattaaaatataatgaaaatggaaccattacagatgctgtagactgtgcacttgaccctctctcagaaacaaagtgtacgttgaaatccttcactgtagaaaaaggaatctatcaaacttctaactttagagtccaaccaacagaatctattgttagatttcctaatattacaaacttgtgcccttttggtgaagtttttaacgccaccagatttgcatctgtttatgcttggaacaggaagagaatcagcaactgtgttgctgattattctgtcctatataattccgcatcattttccacttttaagtgttatggagtgtctcctactaaattaaatgatctctgctttactaatgtctatgcagattcatttgtaattagaggtgatgaagtcagacaaatcgctccagggcaaactggaaatattgctgattataattataaattaccagatgattttacaggctgcgttatagcttggaattctaacaatcttgattctaaggttggtggtaattataattacctgtatagattgtttaggaagtctaatctcaaaccttttgagagagatatttcaactgaaatctatcaggccggtagcacaccttgtaatggtgttaaaggttttaattgttactttcctttacaatcatatggtttccaacccacttatggtgttggttaccaaccatacagagtagtagtactttcttttgaacttctacatgcaccagcaactgtttgtggacctaaaaagtctactaatttggttaaaaacaaatgtgtcaatttcaacttcaatggtttaacaggcacaggtgttcttactgagtctaacaaaaagtttctgcctttccaacaatttggcagagacattgctgacactactgatgctgtccgtgatccacagacacttgagattcttgacattacaccatgttcttttggtggtgtcagtgttataacaccaggaacaaatacttctaaccaggttgctgttctttatcagggtgttaactgcacagaagtccctgttgctattcatgcagatcaacttactcctacttggcgtgtttattctacaggttctaatgtttttcaaacacgtgcaggctgtttaataggggctgaacatgtcaacaactcatatgagtgtgacatacccattggtgcaggtatatgcgctagttatcagactcagactaattctcctcggcgggcacgtagtgtagctagtcaatccatcattgcctacactatgtcacttggtgtagaaaattcagttgcttactctaataactctattgccatacccacaaattttactattagtgttaccacagaaattctaccagtgtctatgaccaagacatcagtagattgtacaatgtacatttgtggtgattcaactgaatgcagcaatcttttgttgcaatatggcagtttttgtacacaattaaaccgtgctttaactggaatagctgttgaacaagacaaaaacacccaagaagtttttgcacaagtcaaacaaatttacaaaacaccaccaattaaagattttggtggttttaatttttcacaaatattaccagatccatcaaaaccaagcaagaggtcatttattgaagatctacttttcaacaaagtgacacttgcagatgctggcttcatcaaacaatatggtgattgccttggtgatattgctgctagagacctcatttgtgcacaaaagtttaacggccttactgttttgccacctttgctcacagatgaaatgattgctcaatacacttctgcactgttagcgggtacaatcacttctggttggacctttggtgcaggtgctgcattacaaataccatttgctatgcaaatggcttataggtttaatggtattggagttacacagaatgttctctatgagaaccaaaaattgattgccaaccaatttaatagtgctattggcaaaattcaagactcactttcttccacagcaagtgcacttggaaaacttcaagatgtggtcaaccaaaatgcacaagctttaaacacgcttgttaaacaacttagctccaattttggtgcaatttcaagtgttttaaatgatatcctttcacgtcttgacaaagttgaggctgaagtgcaaattgataggttgatcacaggcagacttcaaagtttgcagacatatgtgactcaacaattaattagagctgcagaaatcagagcttctgctaatcttgctgctactaaaatgtcagagtgtgtacttggacaatcaaaaagagttgatttttgtggaaagggctatcatcttatgtccttccctcagtcagcacctcatggtgtagtcttcttgcatgtgacttatgtccctgcacaagaaaagaacttcacaactgctcctgccatttgtcatgatggaaaagcacactttcctcgtgaaggtgtctttgtttcaaatggcacacactggtttgtaacacaaaggaatttttatgaaccacaaatcattactacagacaacacatttgtgtctggtaactgtgatgttgtaataggaattgtcaacaacacagtttatgatcctttgcaacctgaattagactcattcaaggaggagttagataaatattttaagaatcatacatcaccagatgttgatttaggtgacatctctggcattaatgcttcagttgtaaacattcaaaaagaaattgaccgcctcaatgaggttgccaagaatttaaatgaatctctcatcgatctccaagaacttggaaagtatgagcagtatataaaatggccatggtacatttggctaggttttatagctggcttgattgccatagtaatggtgacaattatgctttgctgtatgaccagttgctgtagttgtctcaagggctgttgttcttgtggatcctgctgcaaatttgatgaagacgactctgagccagtgctcaaaggagtcaaattacattacacataa

SEQ ID NO: 15 - DNA, 3786 bp, Artificial Sequence
  SARS-CoV-2 spike like protein
atgttcgtgttcctggtgctgctgcctctggtgtccagccagtgcgtgaacttccggaacagaacccagctgcctagcgcctacaccaacagctttaccagaggcgtgtactaccccgacaaggtgttcagatccagcgtgctgcactctacccaggacctgttcctgcctttcttcagcaacgtgacctggttccacgccatcagcggcaccaacgtgatcaagagattcgacaaccccgtgctgcccttcaacgacggggtgtactttgccagcaccgagaagtccaacatcatcagaggctggatcttcggcaccacactggacagcaagacccagagcctgctgatcgtgaacaacgccaccaacgtcgtgatcaaagtgtgcgagttccagttctgcaactaccccttcctgggcgtctaccacaagaacaacaagagctggatggaaagcggcgtgtacagcagcgccaacaactgcaccttcgagtacgtgtcccagcctttcctgatggacctggaaggcaagcagggcaacttcaagaacctgtccgagttcgtgtttaagaacatcgacggctacttcaagatctacagcaagcacacccctatcaacctcgtgcgggatctgcctcagggcttctctgctctggaacccctggtggatctgcccatcggcatcaacatcacccggtttcagacactgctggccctgcacaatagcagctctggatggactgctggcgccgctgcctactatgtgggatacctgcagcctcggaccttcctgctgaagtacaacgagaacggcaccatcaccgacgccgtggattgtgctctggaccctctgagcgagacaaagtgcaccctgaagtccttcaccgtggaaaagggcatctaccagaccagcaacttccgggtgcagcccaccgaatccatcgtgcggttccccaatatcaccaatctgtgccccttcggcgaggtgttcaatgccaccagattcgcctctgtgtacgcctggaaccggaagcggatcagcaattgcgtggccgactactccgtgctgtacaactccgccagcttcagcaccttcaagtgctacggcgtgtcccctaccaagctgaacgacctgtgcttcacaaacgtgtacgccgacagcttcgtgatccggggagatgaagtgcggcagattgcccctggacagacaggcacaatcgccgactacaactacaagctgcccgacgacttcaccggctgtgtgattgcctggaacagcaacaacctggactccaaagtcggcggcaactacaattaccggtacaggctgtttcggaagtccaatctgaagcccttcgagcgggacatctccaccgagatctatcaggccggcagcaagccttgcaatggcgtgcagggcttcaactgctacagcccactgcagagctacggcttccagccaacatacggcgtgggctaccagccttacagagtggtggtgctgagcttcgagctgctgcatgctcctgccacagtgtgcggccctaagaaaagcaccaatctcgtgaagaacaaatgcgtcaacttcaatttcaacggcctgaccggcaccggcgtgctgacagagagcaacaagaagttcctgccattccagcagttcggccgggatatcgccgataccacagatgccgtcagagatccccagacactggaaatcctggacatcaccccttgcagcttcggcggagtgtctgtgatcacccctggcaccaacaccagcaatcaggtggcagtgctgtaccagggcgttaactgtaccgaagtgcccgtggccattcacgccgatcagctgacacctacatggcgggtgtactccaccggctccaacgtgttccagacaagagccggctgtctgatcggagccgagtatgtgaacaacagctacgagtgcgacatccccatcggcgctggcatctgcgcctcttaccagacacagaccaacagcaggcggagagccagatctgtggccagccagagcatcattgcctacacaatgtctctgggcgccgagaacagcgtggcctactccaacaactctatcgctatccccatcaacttcaccatcagcgtgaccacagagatcctgcctgtgtccatgaccaagaccagcgtggactgcaccatgtacatctgcggcgatagcaccgagtgctccaacctgctgctgcagtacggcagcttctgcacccagctgaatagagccctgaccggaatcgccgtggaacaggacaagaacacccaagaggtgttcgcccaagtgaagcagatctacaagacccctcctatcaaggacttcggcggctttaacttcagccagattctgcccgatcctagcaagcccagcaagcggagccctatcgaggacctgctgttcaacaaagtgacactggccgacgccggcttcatcaagcagtatggcgattgtctgggcgacattgccgccagggatctgatttgcgcccagaagttcaacggactgaacgtgctgcctcctctgctgaccgatgagatgatcgcccagtacacatctgccctgctggccggaacaatcaccagcggctggacatttggagctggacccgctctgcagatcccatttccaatgcagatggcctaccggttcaacggcatcggagtgacccagaatgtgctgtacgagaaccagaagctgatcgccaaccagttcaacagcgccatcggcaagatccaggacagcctgagcagcacacctagcgctctgggcaagctgcagaacgtggtcaaccagaatgcccaggcactgaacaccctggtcaagcagctgtccagcaatttcggcgccatctctagcgtgctgaacgatatcctggccagactggacccacctgaggccgaggtgcagatcgacagactgatcacaggacggctgcagtccctgcagacctacgttacacagcagctgatcagagccgccgagattagagcctctgccaatctggccgccatcaagatgagcgagtgtgtgctgggccagagcaagagagtggacttttgcggcaagggctaccacctgatgagcttccctcagtctgctcctcacggcgtggtgtttctgcacgtgacatacgtgcccgctcaagagaagaatttcaccaccgctccagccatctgccacgacggcaaagcccactttcctagagaaggcgtgttcgtgtccaacggcacccattggttcgtgacccagcggaacttctacgagccccagatcatcaccacacacaacaccttcgtgtccggcaactgtgacgttgtgatcggcattgtgaacaataccgtgtacgaccctctgcagcccgagctggactccttcaaagaggaactggacaagtactttaagaaccacacaagccccgacgtggacctgggcgatatcagcggaatcaacgcctccttcgtgaacatccagaaagagatcgaccggctgaacgaggtggccaagaatctgaacgagagcctgatcgacctgcaagaactggggaagtacgagcagtacatcaagtggccttggtacatctggctgggctttatcgccggactgattgccatcgtgatggtcacaatcatgctgtgctgcatgaccagctgctgctcttgcctgaagggctgctgtagctgtggctcctgctgcaagttcgacgaggacgattctgagcccgtgctgaagggcgtgaaactgcactacacatga